European Patent Application EP 4 640 713 A2, published October 29, 2025. Title: ANTIBODY FORMULATIONS. Applicant: SANOFI. Application EP. The sequence listing filed with the application follows.

SEQUENCE LISTING (69 sequences)

SEQ ID NO: 1 - protein, 36 aa, Homo sapiens
MNYPTLEMDLENLEDLFWELDRLDNYNTSLVENHLC

SEQ ID NO: 2 - DNA, 32 bp, synthetic construct
  misc_feature 1..32: note = Description of Artificial Sequence: Synthetic primer
  misc_feature 18: note = n is a, c, g, or t
  source 1..32: mol_type = other DNA
cttccggaattcsargtnmagctgsagsagtc

SEQ ID NO: 3 - DNA, 35 bp, synthetic construct
  misc_feature 1..35: note = Description of Artificial Sequence: Synthetic primer
  misc_feature 18: note = n is a, c, g, or t
  source 1..35: mol_type = other DNA
cttccggaattcsargtnmagctgsagsagtcwgg

SEQ ID NO: 4 - DNA, 36 bp, synthetic construct
  misc_feature 1..36: note = Description of Artificial Sequence: Synthetic primer
  source 1..36: mol_type = other DNA
ggaggatccatagacagatgggggtgtcgttttggc

SEQ ID NO: 5 - DNA, 31 bp, synthetic construct
  misc_feature 1..31: note = Description of Artificial Sequence: Synthetic primer
  source 1..31: mol_type = other DNA
ggagctcgayattgtgmtsacmcarwctmca

SEQ ID NO: 6 - DNA, 46 bp, synthetic construct
  misc_feature 1..46: note = Description of Artificial Sequence: Synthetic primer
  source 1..46: mol_type = other DNA
tatagagctcaagcttggatggtgggaagatggatacagttggtgc

SEQ ID NO: 7 - DNA, 18 bp, synthetic construct
  misc_feature 1..18: note = Description of Artificial Sequence: Synthetic primer
  source 1..18: mol_type = other DNA
ccaagctgtgtcctrtcc

SEQ ID NO: 8 - DNA, 32 bp, synthetic construct
  misc_feature 1..32: note = Description of Artificial Sequence: Synthetic primer
  source 1..32: mol_type = other DNA
cgacaagtcgactagcccttgaccaggcatcc

SEQ ID NO: 9 - DNA, 18 bp, synthetic construct
  misc_feature 1..18: note = Description of Artificial Sequence: Synthetic primer
  source 1..18: mol_type = other DNA
wtctctrgagtcagtggg

SEQ ID NO: 10 - DNA, 32 bp, synthetic construct
  misc_feature 1..32: note = Description of Artificial Sequence: Synthetic primer
  source 1..32: mol_type = other DNA
cgactagtcgactggtgggaagatggatacag

SEQ ID NO: 11 - protein, 112 aa, Mus sp.
DIVMTQAAPSVAVTPRESVSISCRSSKSLLHSSGKTYLYWFLQRPGQSPQLLIYRMSNLASGVPDRFSGSGSGTAFTLRISRVEAEDVGVYYCMQHLEYPYTFGGGTKLEIK

SEQ ID NO: 12 - protein, 111 aa, Mus sp.
QVQLKESGPGLVAPSQSLSITCTVSGFSLIDYGVNWIRQPPGKGLEWLGVIWGDGTTYYNSALKSRLSIRKDNSQSQVFLKMNSLQTDDTAMYYCARIVYWGQGTLVTVSA

SEQ ID NO: 13 - protein, 112 aa, synthetic construct
  REGION 1..112: note = Description of Artificial Sequence: Synthetic polypeptide
DIVMTQSALSVAVTPGESVSISCRSSKSLLHSSGKTYLYWFLQRPGQSPQLLIYRMSNLASGVPDRFSGSGSGTAFTLKISRVEAEDVGVYYCMQHLEYPYTFGGGTKLEIK

SEQ ID NO: 14 - protein, 112 aa, synthetic construct
  REGION 1..112: note = Description of Artificial Sequence: Synthetic polypeptide
DIVMTQSALSVAVTPGESVSISCRSSKSLLHSSGKTYLYWFLQRPGQSPQLLIYRLSNLASGVPDRFSGSGSGTAFTLKISRVEAEDVGVYYCMQHLEYPYTFGGGTKLEIK

SEQ ID NO: 15 - protein, 113 aa, synthetic construct
  REGION 1..113: note = Description of Artificial Sequence: Synthetic polypeptide
DIVMTQSALSVAVTPGESVSISCRSSKSLLHSSGKTYLYWFLQRPGQSPQLLIYRLSSNLASGVPDRFSGSGSGTAFTLKISRVEAEDVGVYYCMQHLEYPYTFGGGTKLEIK

SEQ ID NO: 16 - protein, 111 aa, synthetic construct
  REGION 1..111: note = Description of Artificial Sequence: Synthetic polypeptide
QVQLQESGPGLVAPSESLSITCTVSGFSLIDYGVNWIRQPPGKGLEWLGVIWGDGTTYYNPSLKSRLSISKDNSKSQVFLKMNSLTAADTAMYYCARIVYWGQGTLVTVSS

SEQ ID NO: 17 - protein, 238 aa, synthetic construct
  REGION 1..238: note = Description of Artificial Sequence: Synthetic polypeptide
MGWSCIILFLVATATGVHSDIVMTQSALSVAVTPGESVSISCRSSKSLLHSSGKTYLYWFLQRPGQSPQLLIYRMSNLASGVPDRFSGSGSGTAFTLKISRVEAEDVGVYYCMQHLEYPYTFGGGTKLEIKRTVAAPSVFIFPPSDEQLKSGTASVVCLLNNFYPREAKVQWKVDNALQSGNSQESVTEQDSKDSTYSLSSTLTLSKADYEKHKVYACEVTHQGLSSPVTKSFNRGEC

SEQ ID NO: 18 - DNA, 731 bp, synthetic construct
  misc_feature 1..731: note = Description of Artificial Sequence: Synthetic polynucleotide
  source 1..731: mol_type = other DNA
gctagcaccatgggctggagctgcatcatcctgttcctggtggccaccgccaccggcgtgcacagcgacatcgtgatgacccagagcgccctcagcgtggccgtgacccccggcgagagcgtgagcatcagctgccgcagcagcaagagcctgctgcacagcagcggcaagacctacctgtactggttcctgcagcgccccggccagagcccccagctgctgatctaccgcatgagcaacctggccagcggcgtgcccgaccgcttcagcggcagcggcagcggcaccgccttcaccctgaagatcagccgcgtggaggccgaggacgtgggcgtgtactactgcatgcagcacctggagtacccctacaccttcggcggcggcaccaagctggagatcaagcgtacggtggccgctccttccgtgttcatcttccctccctccgacgagcagctgaagtccggcaccgcctccgtggtgtgtctgctgaacaacttctaccctcgggaggccaaggtgcagtggaaggtggacaacgccctgcagtccggcaactcccaggagtccgtcaccgagcaggactccaaggacagcacctactccctgtcctccaccctgaccctgtccaaggccgactacgagaagcacaaggtgtacgcctgtgaggtgacccaccagggcctgtccagccctgtgaccaagtccttcaaccggggcgagtgctgaagctt

SEQ ID NO: 19 - protein, 238 aa, synthetic construct
  REGION 1..238: note = Description of Artificial Sequence: Synthetic polypeptide
MGWSCIILFLVATATGVHSDIVMTQSALSVAVTPGESVSISCRSSKSLLHSSGKTYLYWFLQRPGQSPQLLIYRLSNLASGVPDRFSGSGSGTAFTLKISRVEAEDVGVYYCMQHLEYPYTFGGGTKLEIKRTVAAPSVFIFPPSDEQLKSGTASVVCLLNNFYPREAKVQWKVDNALQSGNSQESVTEQDSKDSTYSLSSTLTLSKADYEKHKVYACEVTHQGLSSPVTKSFNRGEC

SEQ ID NO: 20 - DNA, 731 bp, synthetic construct
  misc_feature 1..731: note = Description of Artificial Sequence: Synthetic polynucleotide
  source 1..731: mol_type = other DNA
gctagcaccatgggctggagctgcatcatcctgttcctggtggccaccgccaccggcgtgcacagcgacatcgtgatgacccagagcgccctcagcgtggccgtgacccccggcgagagcgtgagcatcagctgccgcagcagcaagagcctgctgcacagcagcggcaagacctacctgtactggttcctgcagcgccccggccagagcccccagctgctgatctaccgcctgagcaacctggccagcggcgtgcccgaccgcttcagcggcagcggcagcggcaccgccttcaccctgaagatcagccgcgtggaggccgaggacgtgggcgtgtactactgcatgcagcacctggagtacccctacaccttcggcggcggcaccaagctggagatcaagcgtacggtggccgctccttccgtgttcatcttccctccctccgacgagcagctgaagtccggcaccgcctccgtggtgtgtctgctgaacaacttctaccctcgggaggccaaggtgcagtggaaggtggacaacgccctgcagtccggcaactcccaggagtccgtcaccgagcaggactccaaggacagcacctactccctgtcctccaccctgaccctgtccaaggccgactacgagaagcacaaggtgtacgcctgtgaggtgacccaccagggcctgtccagccctgtgaccaagtccttcaaccggggcgagtgctgaagctt

SEQ ID NO: 21 - protein, 238 aa, synthetic construct
  REGION 1..238: note = Description of Artificial Sequence: Synthetic polypeptide
MGWSCIILFLVATATGVHSDIVMTQSALSVAVTPGESVSISCRSSKSLLHSSGKTYLYWFLQRPGQSPQLLIYRLSSLASGVPDRFSGSGSGTAFTLKISRVEAEDVGVYYCMQHLEYPYTFGGGTKLEIKRTVAAPSVFIFPPSDEQLKSGTASVVCLLNNFYPREAKVQWKVDNALQSGNSQESVTEQDSKDSTYSLSSTLTLSKADYEKHKVYACEVTHQGLSSPVTKSFNRGEC

SEQ ID NO: 22 - DNA, 731 bp, synthetic construct
  misc_feature 1..731: note = Description of Artificial Sequence: Synthetic polynucleotide
  source 1..731: mol_type = other DNA
gctagcaccatgggctggagctgcatcatcctgttcctggtggccaccgccaccggcgtgcacagcgacatcgtgatgacccagagcgccctcagcgtggccgtgacccccggcgagagcgtgagcatcagctgccgcagcagcaagagcctgctgcacagcagcggcaagacctacctgtactggttcctgcagcgccccggccagagcccccagctgctgatctaccgcctgagcagcctggccagcggcgtgcccgaccgcttcagcggcagcggcagcggcaccgccttcaccctgaagatcagccgcgtggaggccgaggacgtgggcgtgtactactgcatgcagcacctggagtacccctacaccttcggcggcggcaccaagctggagatcaagcgtacggtggccgctccttccgtgttcatcttccctccctccgacgagcagctgaagtccggcaccgcctccgtggtgtgtctgctgaacaacttctaccctcgggaggccaaggtgcagtggaaggtggacaacgccctgcagtccggcaactcccaggagtccgtcaccgagcaggactccaaggacagcacctactccctgtcctccaccctgaccctgtccaaggccgactacgagaagcacaaggtgtacgcctgtgaggtgacccaccagggcctgtccagccctgtgaccaagtccttcaaccggggcgagtgctgaagctt

SEQ ID NO: 23 - protein, 456 aa, synthetic construct
  REGION 1..456: note = Description of Artificial Sequence: Synthetic polypeptide
MGWSCIILFLVATATGVHSQVQLQESGPGLVAPSESLSITCTVSGFSLIDYGVNWIRQPPGKGLEWLGVIWGDGTTYYNPSLKSRLSISKDNSKSQVFLKMNSLTAADTAMYYCARIVYWGQGTLVTVSSASTKGPSVFPLAPCSRSTSESTAALGCLVKDYFPEPVTVSWNSGALTSGVHTFPAVLQSSGLYSLSSVVTVPSSSLGTKTYTCNVDHKPSNTKVDKRVESKYGPPCPSCPAPEFLGGPSVFLFPPKPKDTLMISRTPEVTCVVVDVSQEDPEVQFNWYVDGVEVHNAKTKPREEQFNSTYRVVSVLTVLHQDWLNGKEYKCKVSNKGLPSSIEKTISKAKGQPREPQVYTLPPSQEEMTKNQVSLTCLVKGFYPSDIAVEWESNGQPENNYKTTPPVLDSDGSFFLYSRLTVDKSRWQEGNVFSCSVMHEALHNHYTQKSLSLSLG

SEQ ID NO: 24 - DNA, 1385 bp, synthetic construct
  misc_feature 1..1385: note = Description of Artificial Sequence: Synthetic polynucleotide
  source 1..1385: mol_type = other DNA
gctagcaccatgggctggagctgcatcatcctgttcctggtggccaccgccaccggcgtgcacagccaggtgcagctgcaggagagcggccccggcctggtggcccccagcgagagcctgagcatcacctgcaccgtgagcggcttcagcctgatcgactacggcgtgaactggatccgccagccccccggcaagggcctggagtggctgggcgtgatctggggcgacggcaccacctactacaaccccagcctgaagagccgcctgagcatctccaaggacaacagcaagagccaggtgttcctgaagatgaacagcctgaccgccgccgacaccgccatgtactactgcgcccgcatcgtgtactggggccagggcaccctggtgaccgtgagcagcgccagcaccaagggcccttccgtgttccctctggccccttgctcccggtccacctccgagtccaccgccgctctgggctgcctggtgaaggactacttccctgagcctgtgaccgtgtcctggaactctggcgccctgacctccggcgtgcacaccttccctgccgtgctgcagtcctccggcctgtactccctgtcctccgtggtgaccgtgccttcctcctccctgggcaccaagacctacacctgtaacgtggaccacaagccttccaacaccaaggtggacaagcgggtggagtccaagtacggccctccttgcccttcctgccctgcccctgagttcctgggcggacctagcgtgttcctgttccctcctaagcctaaggacaccctgatgatctcccggacccctgaggtgacctgtgtggtggtggacgtgtcccaggaggaccctgaggtccagttcaactggtacgtggacggcgtggaggtgcacaacgccaagaccaagcctcgggaggagcagttcaattccacctaccgggtggtgtctgtgctgaccgtgctgcaccaggactggctgaacggcaaagaatacaagtgtaaggtctccaacaagggcctgccctcctccatcgagaaaaccatctccaaggccaagggccagcctagggagcctcaggtgtacaccctgcctcctagccaggaagagatgaccaagaaccaggtgtccctgacctgtctggtgaagggcttctacccttccgacatcgccgtggagtgggagtccaacggccagcctgagaacaactacaagaccacccctcctgtgctggactccgacggctccttcttcctgtactccaggctgaccgtggacaagtcccggtggcaggagggcaacgtcttttcctgctccgtgatgcacgaggccctgcacaaccactacacccagaagtccctgtccctgtctctgggctgaagctt

SEQ ID NO: 25 - protein, 22 aa, Homo sapiens
KPGQPPRLLIYDASNRATGIPA

SEQ ID NO: 26 - protein, 12 aa, Mus musculus
TDDTAMYYCARI

SEQ ID NO: 27 - protein, 12 aa, Homo sapiens
SEDSALYYCARD

SEQ ID NO: 28 - protein, 112 aa, Mus musculus; identical to SEQ ID NO: 11

SEQ ID NO: 29 - protein, 111 aa, Mus musculus; identical to SEQ ID NO: 12

SEQ ID NO: 30 - protein, 112 aa, synthetic construct
  REGION 1..112: note = Description of Artificial Sequence: Synthetic polypeptide
DIVMTQAAPSVAVTPGASVSISCRSSKSLLHSSGKTYLYWFLQRPGQSPQLLIYRMSNLASGVPDRFSGSGSGTAFTLRISRVEAEDVGVYYCMQHLEYPYTFGGGTKLEIK

SEQ ID NO: 31 - protein, 112 aa, synthetic construct
  REGION 1..112: note = Description of Artificial Sequence: Synthetic polypeptide
DIVMTQAAPSVAVTPGASVSISCRSSKSLLHSSGKTYLYWFLQRPGQSPQLLIYRLSNLASGVPDRFSGSGSGTAFTLRISRVEAEDVGVYYCMQHLEYPYTFGGGTKLEIK

SEQ ID NO: 32 - protein, 112 aa, synthetic construct
  REGION 1..112: note = Description of Artificial Sequence: Synthetic polypeptide
DIVMTQAAPSVAVTPGASVSISCRSSKSLLHSSGKTYLYWFLQRPGQSPQLLIYRLSSLASGVPDRFSGSGSGTAFTLRISRVEAEDVGVYYCMQHLEYPYTFGGGTKLEIK

SEQ ID NO: 33 - protein, 111 aa, synthetic construct
  REGION 1..111: note = Description of Artificial Sequence: Synthetic polypeptide
QVQLKESGPGLVAPSESLSITCTVSGFSLIDYGVNWIRQPPGKGLEWLGVIWGDGTTYYNPSLKSRLSISKDNSKSQVFLKVTSLTTDDTAMYYCARIVYWGQGTLVTVSA

SEQ ID NO: 34 - protein, 111 aa, synthetic construct
  REGION 1..111: note = Description of Artificial Sequence: Synthetic polypeptide
EVQLKESGPGLVAPGGSLSITCTVSGFSLIDYGVNWIRQPPGKGLEWLGVIWGDGTTYYNAPLKGRLSISKDNSKSQVFLQMNSLKTDDTAMYYCARIVYWGQGTLVTVSS

SEQ ID NO: 35 - protein, 238 aa, synthetic construct
  REGION 1..238: note = Description of Artificial Sequence: Synthetic polypeptide
MGWSCIILFLVATATGVHSDIVMTQAAPSVAVTPRESVSISCRSSKSLLHSSGKTYLYWFLQRPGQSPQLLIYRMSNLASGVPDRFSGSGSGTAFTLRISRVEAEDVGVYYCMQHLEYPYTFGGGTKLEIKRTVAAPSVFIFPPSDEQLKSGTASVVCLLNNFYPREAKVQWKVDNALQSGNSQESVTEQDSKDSTYSLSSTLTLSKADYEKHKVYACEVTHQGLSSPVTKSFNRGEC

SEQ ID NO: 36 - DNA, 731 bp, synthetic construct
  misc_feature 1..731: note = Description of Artificial Sequence: Synthetic polynucleotide
  source 1..731: mol_type = other DNA
gctagcaccatgggctggagctgcatcatcctgttcctggtggccaccgccaccggcgtgcacagcgacatcgtgatgacccaggccgcccccagcgtggccgtgaccccccgcgagagcgtgagcatcagctgccgcagcagcaagagcctgctgcacagcagcggcaagacctacctgtactggttcctgcagcgccccggccagagcccccagctgctgatctaccgcatgagcaacctggccagcggcgtgcccgaccgcttcagcggcagcggcagcggcaccgccttcaccctgcgcatcagccgcgtggaggccgaggacgtgggcgtgtactactgcatgcagcacctggagtacccctacaccttcggcggcggcaccaagctggagatcaagcgtacggtggccgctccttccgtgttcatcttccctccctccgacgagcagctgaagtccggcaccgcctccgtggtgtgtctgctgaacaacttctaccctcgggaggccaaggtgcagtggaaggtggacaacgccctgcagtccggcaactcccaggagtccgtcaccgagcaggactccaaggacagcacctactccctgtcctccaccctgaccctgtccaaggccgactacgagaagcacaaggtgtacgcctgtgaggtgacccaccagggcctgtccagccctgtgaccaagtccttcaaccggggcgagtgctgaagctt

SEQ ID NO: 37 - protein, 456 aa, synthetic construct
  REGION 1..456: note = Description of Artificial Sequence: Synthetic polypeptide
MGWSCIILFLVATATGVHSQVQLKESGPGLVAPSQSLSITCTVSGFSLIDYGVNWIRQPPGKGLEWLGVIWGDGTTYYNSALKSRLSIRKDNSQSQVFLKMNSLQTDDTAMYYCARIVYWGQGTLVTVSAASTKGPSVFPLAPCSRSTSESTAALGCLVKDYFPEPVTVSWNSGALTSGVHTFPAVLQSSGLYSLSSVVTVPSSSLGTKTYTCNVDHKPSNTKVDKRVESKYGPPCPSCPAPEFLGGPSVFLFPPKPKDTLMISRTPEVTCVVVDVSQEDPEVQFNWYVDGVEVHNAKTKPREEQFNSTYRVVSVLTVLHQDWLNGKEYKCKVSNKGLPSSIEKTISKAKGQPREPQVYTLPPSQEEMTKNQVSLTCLVKGFYPSDIAVEWESNGQPENNYKTTPPVLDSDGSFFLYSRLTVDKSRWQEGNVFSCSVMHEALHNHYTQKSLSLSLG

SEQ ID NO: 38 - DNA, 1385 bp, synthetic construct
  misc_feature 1..1385: note = Description of Artificial Sequence: Synthetic polynucleotide
  source 1..1385: mol_type = other DNA
gctagcaccatgggctggagctgcatcatcctgttcctggtggccaccgccaccggcgtgcacagccaggtgcagctgaaggagagcggccccggcctggtggcccccagccagagcctgagcatcacctgcaccgtgagcggcttcagcctgatcgactacggcgtgaactggatccgccagccccccggcaagggcctggagtggctgggcgtgatctggggcgacggcaccacctactacaacagcgccctgaagagccgcctgagcatccgcaaggacaacagccagagccaggtgttcctgaagatgaacagcctgcagaccgacgacaccgccatgtactactgcgcccgcatcgtgtactggggccagggcaccctggtgaccgtgagcgccgccagcaccaagggcccttccgtgttccctctggccccttgctcccggtccacctccgagtccaccgccgctctgggctgcctggtgaaggactacttccctgagcctgtgaccgtgtcctggaactctggcgccctgacctccggcgtgcacaccttccctgccgtgctgcagtcctccggcctgtactccctgtcctccgtggtgaccgtgccttcctcctccctgggcaccaagacctacacctgtaacgtggaccacaagccttccaacaccaaggtggacaagcgggtggagtccaagtacggccctccttgcccttcctgccctgcccctgagttcctgggcggacctagcgtgttcctgttccctcctaagcctaaggacaccctgatgatctcccggacccctgaggtgacctgtgtggtggtggacgtgtcccaggaggaccctgaggtccagttcaactggtacgtggacggcgtggaggtgcacaacgccaagaccaagcctcgggaggagcagttcaattccacctaccgggtggtgtctgtgctgaccgtgctgcaccaggactggctgaacggcaaagaatacaagtgtaaggtctccaacaagggcctgccctcctccatcgagaaaaccatctccaaggccaagggccagcctagggagcctcaggtgtacaccctgcctcctagccaggaagagatgaccaagaaccaggtgtccctgacctgtctggtgaagggcttctacccttccgacatcgccgtggagtgggagtccaacggccagcctgagaacaactacaagaccacccctcctgtgctggactccgacggctccttcttcctgtactccaggctgaccgtggacaagtcccggtggcaggagggcaacgtcttttcctgctccgtgatgcacgaggccctgcacaaccactacacccagaagtccctgtccctgtctctgggctgaagctt

SEQ ID NO: 39 - protein, 238 aa, synthetic construct
  REGION 1..238: note = Description of Artificial Sequence: Synthetic polypeptide
MGWSCIILFLVATATGVHSDIVMTQAAPSVAVTPGASVSISCRSSKSLLHSSGKTYLYWFLQRPGQSPQLLIYRMSNLASGVPDRFSGSGSGTAFTLRISRVEAEDVGVYYCMQHLEYPYTFGGGTKLEIKRTVAAPSVFIFPPSDEQLKSGTASVVCLLNNFYPREAKVQWKVDNALQSGNSQESVTEQDSKDSTYSLSSTLTLSKADYEKHKVYACEVTHQGLSSPVTKSFNRGEC

SEQ ID NO: 40 - DNA, 731 bp, synthetic construct
  misc_feature 1..731: note = Description of Artificial Sequence: Synthetic polypeptide
  source 1..731: mol_type = other DNA
gctagcaccatgggctggagctgcatcatcctgttcctggtggccaccgccaccggcgtgcacagcgacatcgtgatgacccaggccgcccccagcgtggccgtgacccccggcgccagcgtgagcatcagctgccgcagcagcaagagcctgctgcacagcagcggcaagacctacctgtactggttcctgcagcgccccggccagagcccccagctgctgatctaccgcatgagcaacctggccagcggcgtgcccgaccgcttcagcggcagcggcagcggcaccgccttcaccctgcgcatcagccgcgtggaggccgaggacgtgggcgtgtactactgcatgcagcacctggagtacccctacaccttcggcggcggcaccaagctggagatcaagcgtacggtggccgctccttccgtgttcatcttccctccctccgacgagcagctgaagtccggcaccgcctccgtggtgtgtctgctgaacaacttctaccctcgggaggccaaggtgcagtggaaggtggacaacgccctgcagtccggcaactcccaggagtccgtcaccgagcaggactccaaggacagcacctactccctgtcctccaccctgaccctgtccaaggccgactacgagaagcacaaggtgtacgcctgtgaggtgacccaccagggcctgtccagccctgtgaccaagtccttcaaccggggcgagtgctgaagctt

SEQ ID NO: 41 - protein, 238 aa, synthetic construct
  REGION 1..238: note = Description of Artificial Sequence: Synthetic polypeptide
MGWSCIILFLVATATGVHSDIVMTQAAPSVAVTPGASVSISCRSSKSLLHSSGKTYLYWFLQRPGQSPQLLIYRLSNLASGVPDRFSGSGSGTAFTLRISRVEAEDVGVYYCMQHLEYPYTFGGGTKLEIKRTVAAPSVFIFPPSDEQLKSGTASVVCLLNNFYPREAKVQWKVDNALQSGNSQESVTEQDSKDSTYSLSSTLTLSKADYEKHKVYACEVTHQGLSSPVTKSFNRGEC

SEQ ID NO: 42 - DNA, 731 bp, synthetic construct
  misc_feature 1..731: note = Description of Artificial Sequence: Synthetic polynucleotide
  source 1..731: mol_type = other DNA
gctagcaccatgggctggagctgcatcatcctgttcctggtggccaccgccaccggcgtgcacagcgacatcgtgatgacccaggccgcccccagcgtggccgtgacccccggcgccagcgtgagcatcagctgccgcagcagcaagagcctgctgcacagcagcggcaagacctacctgtactggttcctgcagcgccccggccagagcccccagctgctgatctaccgcctgagcaacctggccagcggcgtgcccgaccgcttcagcggcagcggcagcggcaccgccttcaccctgcgcatcagccgcgtggaggccgaggacgtgggcgtgtactactgcatgcagcacctggagtacccctacaccttcggcggcggcaccaagctggagatcaagcgtacggtggccgctccttccgtgttcatcttccctccctccgacgagcagctgaagtccggcaccgcctccgtggtgtgtctgctgaacaacttctaccctcgggaggccaaggtgcagtggaaggtggacaacgccctgcagtccggcaactcccaggagtccgtcaccgagcaggactccaaggacagcacctactccctgtcctccaccctgaccctgtccaaggccgactacgagaagcacaaggtgtacgcctgtgaggtgacccaccagggcctgtccagccctgtgaccaagtccttcaaccggggcgagtgctgaagctt

SEQ ID NO: 43 - protein, 238 aa, synthetic construct
  REGION 1..238: note = Description of Artificial Sequence: Synthetic polypeptide
MGWSCIILFLVATATGVHSDIVMTQAAPSVAVTPGASVSISCRSSKSLLHSSGKTYLYWFLQRPGQSPQLLIYRLSSLASGVPDRFSGSGSGTAFTLRISRVEAEDVGVYYCMQHLEYPYTFGGGTKLEIKRTVAAPSVFIFPPSDEQLKSGTASVVCLLNNFYPREAKVQWKVDNALQSGNSQESVTEQDSKDSTYSLSSTLTLSKADYEKHKVYACEVTHQGLSSPVTKSFNRGEC

SEQ ID NO: 44 - DNA, 731 bp, synthetic construct
  misc_feature 1..731: note = Description of Artificial Sequence: Synthetic polynucleotide
  source 1..731: mol_type = other DNA
gctagcaccatgggctggagctgcatcatcctgttcctggtggccaccgccaccggcgtgcacagcgacatcgtgatgacccaggccgcccccagcgtggccgtgacccccggcgccagcgtgagcatcagctgccgcagcagcaagagcctgctgcacagcagcggcaagacctacctgtactggttcctgcagcgccccggccagagcccccagctgctgatctaccgcctgagcagcctggccagcggcgtgcccgaccgcttcagcggcagcggcagcggcaccgccttcaccctgcgcatcagccgcgtggaggccgaggacgtgggcgtgtactactgcatgcagcacctggagtacccctacaccttcggcggcggcaccaagctggagatcaagcgtacggtggccgctccttccgtgttcatcttccctccctccgacgagcagctgaagtccggcaccgcctccgtggtgtgtctgctgaacaacttctaccctcgggaggccaaggtgcagtggaaggtggacaacgccctgcagtccggcaactcccaggagtccgtcaccgagcaggactccaaggacagcacctactccctgtcctccaccctgaccctgtccaaggccgactacgagaagcacaaggtgtacgcctgtgaggtgacccaccagggcctgtccagccctgtgaccaagtccttcaaccggggcgagtgctgaagctt

SEQ ID NO: 45 - protein, 456 aa, synthetic construct
  REGION 1..456: note = Description of Artificial Sequence: Synthetic polypeptide
MGWSCIILFLVATATGVHSQVQLKESGPGLVAPSESLSITCTVSGFSLIDYGVNWIRQPPGKGLEWLGVIWGDGTTYYNPSLKSRLSISKDNSKSQVFLKVTSLTTDDTAMYYCARIVYWGQGTLVTVSAASTKGPSVFPLAPCSRSTSESTAALGCLVKDYFPEPVTVSWNSGALTSGVHTFPAVLQSSGLYSLSSVVTVPSSSLGTKTYTCNVDHKPSNTKVDKRVESKYGPPCPSCPAPEFLGGPSVFLFPPKPKDTLMISRTPEVTCVVVDVSQEDPEVQFNWYVDGVEVHNAKTKPREEQFNSTYRVVSVLTVLHQDWLNGKEYKCKVSNKGLPSSIEKTISKAKGQPREPQVYTLPPSQEEMTKNQVSLTCLVKGFYPSDIAVEWESNGQPENNYKTTPPVLDSDGSFFLYSRLTVDKSRWQEGNVFSCSVMHEALHNHYTQKSLSLSLG

SEQ ID NO: 46 - DNA, 1385 bp, synthetic construct
  misc_feature 1..1385: note = Description of Artificial Sequence: Synthetic polynucleotide
  source 1..1385: mol_type = other DNA
gctagcaccatgggctggagctgcatcatcctgttcctggtggccaccgccaccggcgtgcacagccaggtgcagctgaaggagagcggccccggcctggtggcccccagcgagagcctgagcatcacctgcaccgtgagcggcttcagcctgatcgactacggcgtgaactggatccgccagccccccggcaagggcctggagtggctgggcgtgatctggggcgacggcaccacctactacaaccccagcctgaagagccgcctgagcatcagcaaggacaacagcaagagccaggtgttcctgaaggtgaccagcctgaccaccgacgacaccgccatgtactactgcgcccgcatcgtgtactggggccagggcaccctggtgaccgtgagcgccgccagcaccaagggcccttccgtgttccctctggccccttgctcccggtccacctccgagtccaccgccgctctgggctgcctggtgaaggactacttccctgagcctgtgaccgtgtcctggaactctggcgccctgacctccggcgtgcacaccttccctgccgtgctgcagtcctccggcctgtactccctgtcctccgtggtgaccgtgccttcctcctccctgggcaccaagacctacacctgtaacgtggaccacaagccttccaacaccaaggtggacaagcgggtggagtccaagtacggccctccttgcccttcctgccctgcccctgagttcctgggcggacctagcgtgttcctgttccctcctaagcctaaggacaccctgatgatctcccggacccctgaggtgacctgtgtggtggtggacgtgtcccaggaggaccctgaggtccagttcaactggtacgtggacggcgtggaggtgcacaacgccaagaccaagcctcgggaggagcagttcaattccacctaccgggtggtgtctgtgctgaccgtgctgcaccaggactggctgaacggcaaagaatacaagtgtaaggtctccaacaagggcctgccctcctccatcgagaaaaccatctccaaggccaagggccagcctagggagcctcaggtgtacaccctgcctcctagccaggaagagatgaccaagaaccaggtgtccctgacctgtctggtgaagggcttctacccttccgacatcgccgtggagtgggagtccaacggccagcctgagaacaactacaagaccacccctcctgtgctggactccgacggctccttcttcctgtactccaggctgaccgtggacaagtcccggtggcaggagggcaacgtcttttcctgctccgtgatgcacgaggccctgcacaaccactacacccagaagtccctgtccctgtctctgggctgaagctt

SEQ ID NO: 47 - protein, 456 aa, synthetic construct
  REGION 1..456: note = Description of Artificial Sequence: Synthetic polypeptide
MGWSCIILFLVATATGVHSEVQLKESGPGLVAPGGSLSITCTVSGFSLIDYGVNWIRQPPGKGLEWLGVIWGDGTTYYNAPLKGRLSISKDNSKSQVFLQMNSLKTDDTAMYYCARIVYWGQGTLVTVSSASTKGPSVFPLAPCSRSTSESTAALGCLVKDYFPEPVTVSWNSGALTSGVHTFPAVLQSSGLYSLSSVVTVPSSSLGTKTYTCNVDHKPSNTKVDKRVESKYGPPCPSCPAPEFLGGPSVFLFPPKPKDTLMISRTPEVTCVVVDVSQEDPEVQFNWYVDGVEVHNAKTKPREEQFNSTYRVVSVLTVLHQDWLNGKEYKCKVSNKGLPSSIEKTISKAKGQPREPQVYTLPPSQEEMTKNQVSLTCLVKGFYPSDIAVEWESNGQPENNYKTTPPVLDSDGSFFLYSRLTVDKSRWQEGNVFSCSVMHEALHNHYTQKSLSLSLG

SEQ ID NO: 48 - DNA, 1385 bp, synthetic construct
  misc_feature 1..1385: note = Description of Artificial Sequence: Synthetic polynucleotide
  source 1..1385: mol_type = other DNA
gctagcaccatgggctggagctgcatcatcctgttcctggtggccaccgccaccggcgtgcacagcgaggtgcagctgaaggagagcggccccggcctggtggcccccggcggcagcctgagcatcacctgcaccgtgagcggcttcagcctgatcgactacggcgtgaactggatccgccagccccccggcaagggcctggagtggctgggcgtgatctggggcgacggcaccacctactacaacgcccccctgaagggccgcctgagcatcagcaaggacaacagcaagagccaggtgttcctgcagatgaacagcctgaagaccgacgacaccgccatgtactactgcgcccgcatcgtgtactggggccagggcaccctggtgaccgtgagcagcgccagcaccaagggcccttccgtgttccctctggccccttgctcccggtccacctccgagtccaccgccgctctgggctgcctggtgaaggactacttccctgagcctgtgaccgtgtcctggaactctggcgccctgacctccggcgtgcacaccttccctgccgtgctgcagtcctccggcctgtactccctgtcctccgtggtgaccgtgccttcctcctccctgggcaccaagacctacacctgtaacgtggaccacaagccttccaacaccaaggtggacaagcgggtggagtccaagtacggccctccttgcccttcctgccctgcccctgagttcctgggcggacctagcgtgttcctgttccctcctaagcctaaggacaccctgatgatctcccggacccctgaggtgacctgtgtggtggtggacgtgtcccaggaggaccctgaggtccagttcaactggtacgtggacggcgtggaggtgcacaacgccaagaccaagcctcgggaggagcagttcaattccacctaccgggtggtgtctgtgctgaccgtgctgcaccaggactggctgaacggcaaagaatacaagtgtaaggtctccaacaagggcctgccctcctccatcgagaaaaccatctccaaggccaagggccagcctagggagcctcaggtgtacaccctgcctcctagccaggaagagatgaccaagaaccaggtgtccctgacctgtctggtgaagggcttctacccttccgacatcgccgtggagtgggagtccaacggccagcctgagaacaactacaagaccacccctcctgtgctggactccgacggctccttcttcctgtactccaggctgaccgtggacaagtcccggtggcaggagggcaacgtcttttcctgctccgtgatgcacgaggccctgcacaaccactacacccagaagtccctgtccctgtctctgggctgaagctt

SEQ ID NO: 49 - protein, 5 aa, Homo sapiens
ELLGG

SEQ ID NO: 50 - protein, 5 aa, Homo sapiens
MISRT

SEQ ID NO: 51 - protein, 6 aa, synthetic construct
  REGION 1..6: note = Description of Artificial Sequence: Synthetic 6x His tag
HHHHHH

SEQ ID NO: 52 - protein, 15 aa, synthetic construct
  REGION 1..15: note = Description of Artificial Sequence: Synthetic peptide
PGKAPQLLIYRMSNL

SEQ ID NO: 53 - protein, 15 aa, synthetic construct
  REGION 1..15: note = Description of Artificial Sequence: Synthetic peptide
PGKAPKLLIYAASSL

SEQ ID NO: 54 - protein, 15 aa, synthetic construct
  REGION 1..15: note = Description of Artificial Sequence: Synthetic peptide
SLIDYGVNWIRQPPG

SEQ ID NO: 55 - protein, 112 aa, synthetic construct
  REGION 1..112: note = Description of Artificial Sequence: Synthetic polypeptide
DIVMTQAAPSVAVTPGQSVSISCRSSKSLLHSSGKTYLYWFLQHPGKAPQLLIYRMSNLASGVPDRFSGSGSGTAFTLTISGVQAEDVGVYYCMQHLEYPYTFGGGTKLEIK

SEQ ID NO: 56 - protein, 113 aa, synthetic construct
  REGION 1..113: note = Description of Artificial Sequence: Synthetic polypeptide
QVQLQESGPGLVAPSQSLSITCTVSGFSLIDYGVNWIRQPPGKGLEWLGVIWGDGTTYYNSALKSRLSISKDTSKSQVFLKMNSLTTDDTAMYYCARIVYWGQGTLVTVSAAK

SEQ ID NO: 57 - protein, 113 aa, synthetic construct
  REGION 1..113: note = Description of Artificial Sequence: Synthetic polypeptide
QVQLQESGPGLVAPSQSLSITCTVSGFSLIDYGVNWIRQPPGKGLEWLGVIWGDGTTYYPSALKSRLSISKDTSKSQVFLKMNSLTTDDTAMYYCARIVYWGQGTLVTVSAAK

SEQ ID NO: 58 - protein, 16 aa, synthetic construct
  REGION 1..16: note = Synthetic peptide
RSSKSLLHSSGKTYLY

SEQ ID NO: 59 - protein, 7 aa, synthetic construct
  REGION 1..7: note = Synthetic peptide
RMSNLAS

SEQ ID NO: 60 - protein, 9 aa, synthetic construct
  REGION 1..9: note = Synthetic peptide
MQHLEYPYT

SEQ ID NO: 61 - protein, 10 aa, synthetic construct
  REGION 1..10: note = Synthetic peptide
GFSLIDYGVN

SEQ ID NO: 62 - protein, 9 aa, synthetic construct
  REGION 1..9: note = Synthetic peptide
VIWGDGTTY

SEQ ID NO: 63 - skipped

SEQ ID NO: 64 - protein, 7 aa, synthetic construct
  REGION 1..7: note = Synthetic peptide
RLSNLAS

SEQ ID NO: 65 - protein, 8 aa, synthetic construct
  REGION 1..8: note = Synthetic peptide
RLSSNLAS

SEQ ID NO: 66 - protein, 6 aa, synthetic construct
  REGION 1..6: note = Synthetic peptide
RMSNLA

SEQ ID NO: 67 - protein, 6 aa, synthetic construct
  REGION 1..6: note = Synthetic peptide
RLSNLA

SEQ ID NO: 68 - protein, 6 aa, synthetic construct
  REGION 1..6: note = Synthetic peptide
RLSSLA

SEQ ID NO: 69 - protein, 17 aa, synthetic construct
  REGION 1..17: note = Synthetic peptide
RSSKSLLHSSGKTYLYW